European Patent Application EP 4 112 634 A1, published January 4, 2023. Title: SARS-COV-2 RECOMBINANT N PROTEIN, AND PREPARATION METHOD AND PURIFICATION METHOD THEREFOR. Applicant: SHENZHEN YHLO BIOTECH CO., LTD. The sequence listing filed with the application follows.

SEQUENCE LISTING (2 sequences)

SEQ ID NO: 1 - protein, 419 aa, artificial sequence
MSDNGPQNQRNAPRITFGGPSDSTGSNQNGERSGARSKQRRPQGLPNNTASWFTALTQHGKEDLKFPRGQGVPINTNSSPDDQIGYYRRATRRIRGGDGKMKDLSPRWYFYYLGTGPEAGLPYGANKDGIIWVATEGALNTPKDHIGTRNPANNAAIVLQLPQGTTLPKGFYAEGSRGGSQASSRSSSRSRNSSRNSTPGSSRGTSPARMAGNGGDAALALLLLDRLNQLESKMSGKGQQQQGQTVTKKSAAEASKKPRQKRTATKAYNVTQAFGRRGPEQTQGNFGDQELIRQGTDYKHWPQIAQFAPSASAFFGMSRIGMEVTPSGTWLTYTAAIKLDDKDPNFKDQVILLNKHIDAYKTFPPTEPKKDKKKKADETQALPQRQKKQQTVTLLPAADLDDFSKQLQQSMSSADSTQA

SEQ ID NO: 2 - DNA, 1317 bp, artificial sequence
atgcgtcgcagacgtcgaggatctggctcgatgagtgataacggcccgcagaatcagcgcaatgccccgcgcattacctttggtggcccgagtgatagtaccggtagtaatcagaatggtgaacgcagcggcgcccgcagtaaacagcgtcgtccgcagggtctgccgaataataccgcaagctggtttaccgccctgacccagcatggcaaagaagatctgaaatttccgcgcggtcagggtgttccgattaataccaatagcagtccggatgatcagattggttattatcgtcgtgccacccgtcgtattcgcggcggcgatggtaaaatgaaagatctgagtccgcgttggtatttttattatctgggcaccggtccggaagcaggcctgccttatggtgccaataaggatggcattatttgggtggcaaccgaaggcgccctgaataccccgaaagatcatattggtacccgtaatccggccaataatgcagcaattgtgctgcagctgccgcagggcaccaccctgcctaaaggcttttatgcagaaggtagtcgcggtggcagccaggcaagcagccgtagtagtagccgcagtcgtaatagcagtcgcaatagcaccccgggtagcagtcgtggtaccagcccggcacgcatggcaggcaatggtggtgacgccgcactggcactgctgctgctggatcgtctgaatcagctggaaagcaaaatgagtggcaaaggtcagcagcagcagggccagaccgtgaccaaaaaatctgccgcagaagccagcaaaaaaccgcgtcagaaacgtaccgccaccaaagcctataatgtgacccaggcatttggccgtcgcggcccggaacagacccagggtaattttggtgaccaggaactgattcgccagggcaccgattataaacattggccgcagattgcacagtttgcaccgagtgccagtgcctttttcggcatgagccgcattggcatggaagttaccccgagtggtacctggctgacctataccggtgccattaagctggatgataaagatccgaattttaaagatcaggttattctgctgaacaaacatattgatgcctataaaaccttcccgccgaccgaaccgaaaaaagataaaaagaaaaaggcagatgagacccaggcactgccgcagcgccagaaaaaacagcagaccgtgacactgctgccggcagcagatctggatgattttagtaaacagctgcagcagagcatgagtagcgccgatagtacccaggccggatctggctcgcgtcgcagacgtcgataa